European Patent Application EP 4 154 904 A1, published March 29, 2023. Title: COMPOSITIONS AND METHODS FOR INCREASING OR ENHANCING TRANSDUCTION OF GENE THERAPY VECTORS AND FOR REMOVING OR REDUCING IMMUNOGLOBULINS. Applicant: INSTITUT NATIONAL DE LA SANTE ET DE LA RECHERCHE MEDICALE (INSERM). Application EP. The sequence listing filed with the application follows.

SEQUENCE LISTING (52 sequences)

SEQ ID NO: 1 - protein, 738 aa, synthetic construct
  REGION 1..738: note = Spk1
MAADGYLPDWLEDNLSEGIREWWDLKPGAPKPKANQQKQDNGRGLVLPGYKYLGPFNGLDKGEPVNAADAAALEHDKAYDQQLQAGDNPYLRYNHADAEFQERLQEDTSFGGNLGRAVFQAKKRVLEPLGLVESPVKTAPGKKRPVEPSPQRSPDSSTGIGKKGQQPAKKRLNFGQTGDSESVPDPQPIGEPPAAPSGVGPNTMAAGGGAPMADNNEGADGVGSSSGNWHCDSTWLGDRVITTSTRTWALPTYNNHLYKQISNGTSGGSTNDNTYFGYSTPWGYFDFNRFHCHFSPRDWQRLINNNWGFRPKRLNFKLFNIQVKEVTQNEGTKTIANNLTSTIQVFTDSEYQLPYVLGSAHQGCLPPFPADVFMIPQYGYLTLNNGSQAVGRSSFYCLEYFPSQMLRTGNNFEFSYNFEDVPFHSSYAHSQSLDRLMNPLIDQYLYYLSRTQSTGGTAGTQQLLFSQAGPNNMSAQAKNWLPGPCYRQQRVSTTLSQNNNSNFAWTGATKYHLNGRDSLVNPGVAMATHKDDEERFFPSSGVLMFGKQGAGKDNVDYSSVMLTSEEEIKTTNPVATEQYGVVADNLQQQNAAPIVGAVNSQGALPGMVWQNRDVYLQGPIWAKIPHTDGNFHPSPLMGGFGLKHPPPQILIKNTPVPADPPTTFNQAKLASFITQYSTGQVSVEIEWELQKENSKRWNPEIQYTSNYYKSTNVDFAVNTEGTYSEPRPIGTRYLTRNL

SEQ ID NO: 2 - protein, 736 aa, synthetic construct
  REGION 1..736: note = Spk2
MAADGYLPDWLEDNLSEGIREWWALQPGAPKPKANQQHQDNARGLVLPGYKYLGPGNGLDKGEPVNAADAAALEHDKAYDQQLKAGDNPYLKYNHADAEFQERLKEDTSFGGNLGRAVFQAKKRLLEPLGLVEEAAKTAPGKKRPVDQSPQEPDSSSGVGKSGKQPARKRLNFGQTGDSESVPDPQPLGEPPAAPTSLGSNTMASGGGAPMADNNEGADGVGNSSGNWHCDSQWLGDRVITTSTRTWALPTYNNHLYKQISSQSGASNDNHYFGYSTPWGYFDFNRFHCHFSPRDWQRLINNNWGFRPKKLSFKLFNIQVKEVTQNDGTTTIANNLTSTVQVFTDSEYQLPYVLGSAHQGCLPPFPADVFMVPQYGYLTLNNGSQAVGRSSFYCLEYFPSQMLRTGNNFQFSYTFEDVPFHSSYAHSQSLDRLMNPLIDQYLYYLNRTQGTTSGTTNQSRLLFSQAGPQSMSLQARNWLPGPCYRQQRLSKTANDNNNSNFPWTAASKYHLNGRDSLVNPGPAMASHKDDEEKFFPMHGNLIFGKEGTTASNAELDNVMITDEEEIRTTNPVATEQYGTVANNLQSSNTAPTTRTVNDQGALPGMVWQDRDVYLQGPIWAKIPHTDGHFHPSPLMGGFGLKHPPPQIMIKNTPVPANPPTTFSPAKFASFITQYSTGQVSVEIEWELQKENSKRWNPEIQYTSNYNKSVNVDFTVDTNGVYSEPRPIGTRYLTRPL

SEQ ID NO: 3 - protein, 339 aa, Streptococcus pyogenes
MRKRCYSTSAAVLAAVTLFVLSVDRGVIADSFSANQEIRYSEVTPYHVTSVWTKGVTPPANFTQGEDVFHAPYVANQGWYDITKTFNGKDDLLCGAATAGNMLHWWFDQNKDQIKRYLEEHPEKQKINFNGEQMFDVKEAIDTKNHQLDSKLFEYFKEKAFPYLSTKHLGVFPDHVIDMFINGYRLSLTNHGPTPVKEGSKDPRGGIFDAVFTRGDQSKLLTSRHDFKEKNLKEISDLIKKELTEGKALGLSHTYANVRINHVINLWGADFDSNGNLKAIYVTDSDSNASIGMKKYFVGVNSAGKVAISAKEIKEDNIGAQVLGLFTLSTGQDSWNQTN

SEQ ID NO: 4 - protein, 310 aa, Streptococcus pyogenes
DSFSANQEIRYSEVTPYHVTSVWTKGVTPPANFTQGEDVFHAPYVANQGWYDITKTFNGKDDLLCGAATAGNMLHWWFDQNKDQIKRYLEEHPEKQKINFNGEQMFDVKEAIDTKNHQLDSKLFEYFKEKAFPYLSTKHLGVFPDHVIDMFINGYRLSLTNHGPTPVKEGSKDPRGGIFDAVFTRGDQSKLLTSRHDFKEKNLKEISDLIKKELTEGKALGLSHTYANVRINHVINLWGADFDSNGNLKAIYVTDSDSNASIGMKKYFVGVNSAGKVAISAKEIKEDNIGAQVLGLFTLSTGQDSWNQTN

SEQ ID NO: 5 - protein, 310 aa, Streptococcus pyogenes
DSFSANQEIRYSEVTPYHVTSVWTKGVTPPANFTQGEDVFHAPYVANQGWYDITKTFNGKDDLLCGAATAGNMLHWWFDQNKDQIKRYLEEHPEKQKINFRGEQMFDVKEAIDTKNHQLDSKLFEYFKEKAFPYLSTKHLGVFPDHVIDMFINGYRLSLTNHGPTPVKEGSKDPRGGIFDAVFTRGDQSKLLTSRHDFKEKNLKEISDLIKKELTEGKALGLSHTYANVRINHVINLWGADFDSNGNLKAIYVTDSDSNASIGMKKYFVGVNSAGKVAISAKEIKEDNIGAQVLGLFTLSTGQDSWNQTN

SEQ ID NO: 6 - protein, 310 aa, Streptococcus pyogenes
DSFSANQEIRYSEVTPYHVTSVWTKGVTPPANFTQGEDVFHAPYVANQGWYDITKTFNGKDDLLCGAATAGNMLHWWFDQNKDQIKRYLEEHPEKQKINFKGEQMFDVKEAIDTKNHQLDSKLFEYFKEKAFPYLSTKHLGVFPDHVIDMFINGYRLSLTNHGPTPVKRGSKDPRGGIFDAVFTRGNQSKLLTSRHDFKEKNLKEISDLIKKELTEGKALGLSHTYANVRINHVINLWGADFDSNGNLKAIYVTDSDSNASIGMKKYFVGVNSAGKVAISAKEIKEDNIGAQVLGLFTLSTGQDSWNQTN

SEQ ID NO: 7 - protein, 310 aa, Streptococcus pyogenes
DSFSANQEIRYSEVTPYHVTSVWTKGVTPPANFTQGEDVFHAPYVANQGWYDITKTFNGKDDLLCGAATAGNMLHWWFDQNKDQIKRYLEEHPEKQKINFRGEQMFDVKEAIDTKNHQLDSKLFEYFKEKAFPYLSTKHLGVFPDHVIDMFINGYRLSLTNHGPTPVKKGSKDPRGGIFDAVFTRGNQSKLLTSRHDFKEKNLKEISDLIKKELTEGKALGLSHTYANVRINHVINLWGADFDSNGNLKAIYVTDSDSNASIGMKKYFVGVNKAGKVAISAKEIKEDNIGAQVLGLFTLSTGQDSWNQTN

SEQ ID NO: 8 - protein, 310 aa, Streptococcus pyogenes
DSFSANQEIRYSEVTPYHVTSVWTKGVTPPANFTQGEDVFHAPYVANQGWYDITKTFNGKDDLLCGAATAGNMLHWWFDQNKDQIKRYLREHPEKQKINFNGEQMFDVKEAIDTKNHQLDSKLFEYFKEKAFPYLSTKHLGVFPDHVIDMFINGYRLSLTNHGPTPVKEGSKDPRGGIFDAVFTRGNQSKLLTSRHDFKEKNLKEISDLIKKELDEGKALGLSHTYANVRINHVINLWGADFDSNGNLKAIYVTDSDSNASIGMKKYFVGVNSAGKVAISAKEIKEDNIGAQVLGLFTLSTGQDSWNQTN

SEQ ID NO: 9 - protein, 310 aa, Streptococcus pyogenes
DSFSANQEIRYSEVTPYHVTSVWTKGVTPPANFTQGEDVFHAPYVANQGWYDITKTFNGKDDLLCGAATAGNMLHWWFDQNKDQIKRYLKEHPEKQKINFNGEQMFDVKEAIRTKNHQLDSKLFEYFKEKAFPYLSTKHLGVFPDHVIDMFINGYRLSLTNHGPTPVKEGSKDPRGGIFDAVFTRGNQSKLLTSRHDFKEKNLKEISDLIKKELEEGKALGLSHTYANVRINHVINLWGADFDSNGNLKAIYVTDSDSNASIGMKKYFVGVNKAGKVAISAKEIKEDNIGAQVLGLFTLSTGQDSWNQTN

SEQ ID NO: 10 - protein, 310 aa, Streptococcus pyogenes
DSFSANQEIRYSEVTPYHVTSVWTKGVTPPANFTQGEDVFHAPYVANQGWYDITKTFNGKDDLLCGAATAGNMLHWWFDQNKDQIERYLEEHPEKQKINFNGEQMFDVKEAIDTKNHQLDSKLFEYFKEKAFPYLSTKHLGVFPDHVIDMFINGYRLSLTNHGPTPVKEGSKDPRGGIFDAVFTRGNQSKLLTSRHDFKEKNLKEISDLIKEELTKGKALGLSHTYANVRINHVINLWGADFDSNGNLKAIYVTDSDSNASIGMKKYFVGVNSAGKVAISAKEIKEKNIGAQVLGLFTLSTGQKSWNQTN

SEQ ID NO: 11 - protein, 310 aa, Streptococcus pyogenes
DSFSANQEIRYSEVTPYHVTSVWTKGVTPPANFTQGEDVFHAPYVANQGWYDITKTFNGKDDLLCGAATAGNMLHWWFDQNKDQIKRYLKEHPEKQKINFRGEQMFDVKEAIRTKNHQLDSKLFEYFKEKAFPYLSTKHLGVFPDHVIDMFINGYRLSLTNHGPTPVKEGSKDPRGGIFDAVFTRGNQSKLLTSRHDFKEKNLKEISDLIKSELENGKALGLSHTYANVRINHVINLWGADFDSNGNLKAIYVTDSDSNASIGMKKYFVGVNKAGKVAISAKEIKEDNIGAQVLGLFTLSTGQDSWNQTN

SEQ ID NO: 12 - protein, 310 aa, Streptococcus pyogenes
DSFSANQEIRYSEVTPYHVTSVWTKGVTPPANFTQGEDVFHAPYVANQGWYDITKTFNGKDDLLCGAATAGNMLHWWFDQNKDQIKRYLKEHPEKQKINFRGEQMFDVKEAIRTKNHQLDSKLFEYFKEKAFPYLSTKHLGVFPDHVIDMFINGYRLSLTNHGPTPVKKGSKDPRGGIFDAVFTRGNQSKLLTSRHDFKEKNLKEISDLIKKELEEGKALGLSHTYANVRINHVINLWGADFDSNGNLKAIYVTDSDSNASIGMKKYFVGVNSAGKVAISAKEIKEDNIGAQVLGLFTLSTGQDSWNQTN

SEQ ID NO: 13 - protein, 310 aa, Streptococcus pyogenes
DSFSANQEIRYSEVTPYHVTSVWTKGVTPPANFTQGEDVFHAPYVANQGWYDITKTFNGKDDLLCGAATAGNMLHWWFDQNKDQIERYLEEHPEKQKINFRGEQMFDVKEAIDTKNHQLDSKLFEYFKEKAFPYLSTKHLGVFPDHVIDMFINGYRLSLTNHGPTPVKKGSKDPRGGIFDAVFTRGNQSKLLTSRHDFKEKNLKEISDLIKEELTKGKALGLSHTYANVRINHVINLWGADFDSNGNLKAIYVTDSDSNASIGMKKYFVGVNSAGKVAISAKEIKEDNIGAQVLGLFTLSTGQKSWNQTN

SEQ ID NO: 14 - protein, 306 aa, Streptococcus pyogenes
DSFSANQEIRYSEVTPYHVTSVWTKGVTPPANFTQGEDVFHAPYVANQGWYDITKTFNGKDDLLCGAATAGNMLHWWFDQNKDQIKRYLEEHPEKQKINFNGEQMFDVKEAIDTKNHQLDSKLFEYFKEKAFPYLSTKHLGVFPDHVIDMFINGYRLSLTNHGPTPVKEGSKDPRGGIFDAVFTRGDQSKLLTSRHDFKEKNLKEISDLIKKELTEGKALGLSHTYANVRINHVINLWGADFDSNGNLKAIYVTDSDSNASIGMKKYFVGVNSAGKVAISAKEIKEDNIGAQVLGLFTLSTGQDSW

SEQ ID NO: 15 - protein, 290 aa, Streptococcus pyogenes
SVWTKGVTPPANFTQGEDVFHAPYVANQGWYDITKTFNGKDDLLCGAATAGNMLHWWFDQNKDQIKRYLEEHPEKQKINFNGEQMFDVKEAIDTKNHQLDSKLFEYFKEKAFPYLSTKHLGVFPDHVIDMFINGYRLSLTNHGPTPVKEGSKDPRGGIFDAVFTRGDQSKLLTSRHDFKEKNLKEISDLIKKELTEGKALGLSHTYANVRINHVINLWGADFDSNGNLKAIYVTDSDSNASIGMKKYFVGVNSAGKVAISAKEIKEDNIGAQVLGLFTLSTGQDSWNQTN

SEQ ID NO: 16 - protein, 290 aa, Streptococcus pyogenes
SVWTKGVTPPANFTQGEDVFHAPYVANQGWYDITKTFNGKDDLLCGAATAGNMLHWWFDQNKDQIKRYLEEHPEKQKINFKGEQMFDVKEAIDTKNHQLDSKLFEYFKEKAFPYLSTKHLGVFPDHVIDMFINGYRLSLTNHGPTPVKEGSKDPRGGIFDAVFTRGNQSKLLTSRHDFKEKNLKEISDLIKKELTEGKALGLSHTYANVRINHVINLWGADFDSNGNLKAIYVTDSDSNASIGMKKYFVGVNSAGKVAISAKEIKEDNIGAQVLGLFTLSTGQDSWNQTN

SEQ ID NO: 17 - protein, 290 aa, Streptococcus pyogenes
SVWTKGVTPPANFTQGEDVFHAPYVANQGWYDITKTFNGKDDLLCGAATAGNMLHWWFDQNKDQIERYLEEHPEKQKINFKGEQMFDVKKAIDTKNHQLDSKLFEYFKEKAFPYLSTKHLGVFPDHVIDMFINGYRLSLTNHGPTPVKEGSKDPRGGIFDAVFTRGNQSKLLTSRHDFKEKNLKEISDLIKEELTKGKALGLSHTYANVRINHVINLWGADFDSNGNLKAIYVTDSDSNASIGMKKYFVGVNSAGKVAISAKEIKEDNIGAQVLGLFTLSTGQKSWNQTN

SEQ ID NO: 18 - protein, 319 aa, Streptococcus pyogenes
DDYQRNATEAYAKEVPHQITSVWTKGVTPPANFTQGEDVFHAPYVANQGWYDITKTFNGKDDLLCGAATAGNMLHWWFDQNKDQIERYLEEHPEKQKINFKGEQMFDVKKAIDTKNHQLDSKLFEYFKEKAFPYLSTKHLGVFPDHVIDMFINGYRLSLTNHGPTPVKEGSKDPRGGIFDAVFTRGNQSKLLTSRHDFKEKNLKEISDLIKEELTKGKALGLSHTYANVRINHVINLWGADFDSNGNLKAIYVTDSDSNASIGMKKYFVGVNSAGKVAISAKEIKEDNIGAQVLGLFTLSTGQKSWNQTNGGGHHHHHH

SEQ ID NO: 19 - protein, 586 aa, Streptococcus agalactiae
NQNNIQETNLVEKNSEDKFIQELNRYKTEIPNFKGFNVWILGDKGYYKNLINLEEIKNIQATLKKERNEEYVFVKLNGKIAHDTTVFLMNKKHKLLKNIEEFKTITQKRLTERGKFPYDTVHSTFEIKDENFIMERLKSSGLSMGKPVDYMGVNGIPIYTKTLSIDNKFAFENNSKDSSYSSNINISEDKIKENDQKILDLIVKSGANNQNLTDEEKVIAFTKYIGEITNYDNEAYRARNVDTEYYRASDLFSVTERKLAMCVGYSVTAARAFNIMGIPSYVVSGKSPQGISHAAVRAYYNRSWHIIDITASTYWKNGNYKTTYSDFIKEYCIDGYDVYDPAKTNNRFKVKYMESNEAFENWIHNNGSKSMLFINESAALKDKKPKDDFVPVTEKEKNELIDKYKKLLSQIPENTQNPGEKNIRDYLKNEYEEILKKDNLFEHEHAEFKESLNLNESFYLQLKKEEKKPSDNLKKEEKPRENSVKERETPAENNDFVSVTEKNNLIDKYKELLSKIPENTQNPGEKNIRNYLEKEYEELLQKDKLFKHEYTEFTKSLNLNETFYSQLKEGEMKLSENPEKGETNTN

SEQ ID NO: 20 - protein, 497 aa, Streptococcus pseudoporcinus
RENENVRQLQSENKQMKAVNLQEFSEKLKGEIAENQQFHIFKLGLNNYYIGGVRINELSDLAKNHDFIMIDNRATHNKYGVPHIIIMNKDDVIVHNQEDYNKEMAELTFAGDKPIQSDSYLPQKKRIHALFEIGLDSNRRQLLNAAGLKTPENSVIELDTFKIYSHGLAVDNKYYDEYSHFNNNTNVNITKQRFTENDNLIHNLITTSTAKDQPTDRDKVKTFVMYVANHTIYDWNAANNAVSNISDVNYYLGSDLFSITERKKAMCVGFSTTAARAFNMLGIPAYVVEGKNAQGVDHATARVYYNGKWHTIDGTGFINGNRTRSTLYTESHFRSVGEDSYQLVGLNEDIPFDRNYMKIDKVYEEWAPKQKTADLLLVNKDKSLVGLDRVAYVEPVYVDKNRQDALTQIYKKLKETMESSSKKNPSSGGFSSLLGSASSDIAKLEGSSQLTQEEYDKIHRSMTSILTFFAQLDKDAAEAFEKGNDYKNYLATTKHAQ

SEQ ID NO: 21 - protein, 349 aa, Streptococcus equi
MKTIAYPNKPHSLSAGLLTAIAIFSLASSNITYADDYQRNATEAYAKEVPHQITSVWTKGVTPLTPEQFRYNNEDVIHAPYLAHQGWYDITKAFDGKDNLLCGAATAGNMLHWWFDQNKTEIEAYLSKHPEKQKIIFNNQELFDLKAAIDTKDSQTNSQLFNYFRDKAFPNLSARQLGVMPDLVLDMFINGYYLNVFKTQSTDVNRPYQDKDKRGGIFDAVFTRGDQTTLLTARHDLKNKGLNDISTIIKQELTEGRALALSHTYANVSISHVINLWGADFNAEGNLEAIYVTDSDANASIGMKKYFVGINAHGHVAISAKKIEGENIGAQVLGLFTLSSGKDIWQKLS

SEQ ID NO: 22 - protein, 315 aa, Streptococcus equi
DDYQRNATEAYAKEVPHQITSVWTKGVTPLTPEQFRYNNEDVIHAPYLAHQGWYDITKAFDGKDNLLCGAATAGNMLHWWFDQNKTEIEAYLSKHPEKQKIIFNNQELFDLKAAIDTKDSQTNSQLFNYFRDKAFPNLSARQLGVMPDLVLDMFINGYYLNVFKTQSTDVNRPYQDKDKRGGIFDAVFTRGDQTTLLTARHDLKNKGLNDISTIIKQELTEGRALALSHTYANVSISHVINLWGADFNAEGNLEAIYVTDSDANASIGMKKYFVGINAHGHVAISAKKIEGENIGAQVLGLFTLSSGKDIWQKLS

SEQ ID NO: 23 - protein, 313 aa, synthetic construct
  REGION 1..313: note = IdeS/Z hybrid
DDYQRNATEAYAKEVPHQITSVWTKGVTPLTPEQFRYNNEDVFHAPYVANQGWYDITKAFDGKDNLLCGAATAGNMLHWWFDQNKDQIKRYLEEHPEKQKINFNGDNMFDVKKAIDTKNHQLDSKLFNYFKEKAFPGLSARRIGVFPDHVIDMFINGYRLSLTNHGPTPVKEGSKDPRGGIFDAVFTRGNQSKLLTSRHDFKNKNLNDISTIIKQELTKGKALGLSHTYANVSINHVINLWGADFNAEGNLEAIYVTDSDSNASIGMKKYFVGVNAHGHVAISAKKIEGENIGAQVLGLFTLSTGQDSWQKLS

SEQ ID NO: 24 - protein, 315 aa, Streptococcus equi
DDYQRNATEAYAKEVPHQITSVWTKGVTPLTPEQFRYNNEDVIHAPYLANQGWYDITKAFDGKDNLLCGAATAGNMLHWWFDQNKTEIEAYLSKHPEKQKIIFRNQELFDLKEAIRTKDSQTNSQLFEYFRDKAFPYLSARQLGVMPDLVLDMFINGYYLNVFKTQSTDVKRPYQDKDKRGGIFDAVFTRGNQTTLLTARHDLKNKGLNDISTIIKEELTKGRALALSHTYANVSISHVINLWGADFNAEGNLEAIYVTDSDANASIGMKKYFVGINKHGHVAISAKKIEGENIGAQVLGLFTLSSGKDIWQKLN

SEQ ID NO: 25 - protein, 315 aa, Streptococcus equi
DDYQRNATEAYAKEVPHQITSVWTKGVTPLTPEQFRYNNEDVIHAPYLAHQGWYDITKTFNGKDNLLCGAATAGNMLHWWFDQNKTEIEAYLSKHPEKQKIIFNNEELFDLKAAIDTKDSQTNSQLFNYFKEKAFPNLSTRQLGVMPDLVLDMFINGYYLNVFKTQSTDVNRPYQDKDKRGGIFDAVFTRGNQTTLLTARHDFKEKGLKDISTIIKQELTEGRALALSHTYANVSISHVINLWGADFDAEGNLKAIYVTDSDANASIGMKKYFVGINAHGKVAISAKKIEGENIGAQVLGLFTLSSGKDIWQQLS

SEQ ID NO: 26 - protein, 315 aa, Streptococcus equi
DSFSANQEIRYSEVTPYHVTSVWTKGVTPLTPEQFRYNNEDVIHAPYLAHQGWYDITKAFDGKDNLLCGAATAGNMLHWWFDQNKTEIEAYLSKHPEKQKIIFNNQELFDLKAAIDTKDSQTNSQLFNYFRDKAFPNLSARQLGVMPDLVLDMFINGYYLNVFKTQSTDVNRPYQDKDKRGGIFDAVFTRGDQTTLLTARHDLKNKGLNDISTIIKQELTEGRALALSHTYANVSISHVINLWGADFNAEGNLEAIYVTDSDANASIGMKKYFVGINAHGHVAISAKKIEGENIGAQVLGLFTLSSGKDIWQKLS

SEQ ID NO: 27 - protein, 295 aa, Streptococcus equi
SVWTKGVTPLTPEQFRYNNEDVIHAPYLAHQGWYDITKAFDGKDNLLCGAATAGNMLHWWFDQNKTEIEAYLSKHPEKQKIIFNNQELFDLKAAIDTKDSQTNSQLFNYFRDKAFPNLSARQLGVMPDLVLDMFINGYYLNVFKTQSTDVNRPYQDKDKRGGIFDAVFTRGDQTTLLTARHDLKNKGLNDISTIIKQELTEGRALALSHTYANVSISHVINLWGADFNAEGNLEAIYVTDSDANASIGMKKYFVGINAHGHVAISAKKIEGENIGAQVLGLFTLSSGKDIWQKLS

SEQ ID NO: 28 - protein, 314 aa, Streptococcus equi
DDYQRNATEAYAKEVPHQITSVWTKGVTPLTPEQFTQGEDVIHAPYLAHQGWYDITKAFDGKDNLLCGAATAGNMLHWWFDQNKTEIEAYLSKHPEKQKIIFNNQELFDLKAAIDTKDSQTNSQLFNYFRDKAFPNLSARQLGVMPDLVLDMFINGYYLNVFKTQSTDVNRPYQDKDKRGGIFDAVFTRGDQTTLLTARHDLKNKGLNDISTIIKQELTEGRALALSHTYANVSISHVINLWGADFNAEGNLEAIYVTDSDANASIGMKKYFVGINAHGHVAISAKKIEGENIGAQVLGLFTLSSGKDIWQKLS

SEQ ID NO: 29 - protein, 312 aa, Streptococcus equi
DDYQRNATEAYAKEVPHQITSVWTKGVTPPEQFTQGEDVIHAPYLAHQGWYDITKAFDGKDNLLCGAATAGNMLHWWFDQNKTEIEAYLSKHPEKQKIIFNNQELFDLKAAIDTKDSQTNSQLFNYFRDKAFPNLSARQLGVMPDLVLDMFINGYYLNVFKTQSTDVNRPYQDKDKRGGIFDAVFTRGDQTTLLTARHDLKNKGLNDISTIIKQELTEGRALALSHTYANVSISHVINLWGADFNAEGNLEAIYVTDSDANASIGMKKYFVGINAHGHVAISAKKIEGENIGAQVLGLFTLSSGKDIWQKLS

SEQ ID NO: 30 - protein, 313 aa, Streptococcus equi
DDYQRNATEAYAKEVPHQITSVWTKGVTPPEQFRYNNEDVIHAPYLAHQGWYDITKAFDGKDNLLCGAATAGNMLHWWFDQNKTEIEAYLSKHPEKQKIIFNNQELFDLKAAIDTKDSQTNSQLFNYFRDKAFPNLSARQLGVMPDLVLDMFINGYYLNVFKTQSTDVNRPYQDKDKRGGIFDAVFTRGDQTTLLTARHDLKNKGLNDISTIIKQELTEGRALALSHTYANVSISHVINLWGADFNAEGNLEAIYVTDSDANASIGMKKYFVGINAHGHVAISAKKIEGENIGAQVLGLFTLSSGKDIWQKLS

SEQ ID NO: 31 - protein, 312 aa, Streptococcus equi
DDYQRNATEAYAKEVPHQITSVWTKGVTPPEQFTQGEDVIHAPYLAHQGWYDITKAFDGKDNLLCGAATAGNMLHWWFDQNKTEIEAYLSKHPEKQKIIINNQELFDLKAAIDTKDSQTNSQLFNYFRDKAFPNLSARQLGVMPDLVLDMFINGYYLNVFKTQSTDVNRPYQDKDKRGGIFDAVFTRGDQTTLLTARHDLKNKGLNDISTIIKQELTEGRALALSHTYANVSISHVINLWGADFNAEGNLEAIYVTDSDANASIGMKKYFVGINAHGHVAISAKKIEGENIGAQVLGLFTLSSGKDIWQKLS

SEQ ID NO: 32 - protein, 312 aa, Streptococcus equi
DDYQRNATEAYAKEVPHQITSVWTKGVTPPEQFTQGEDVIHAPYLAHQGWYDITKAFDGKDNLLCGAATAGNMLHWWFDQNKTEIEAYLSKHPEKQKIIFRNQELFDLKAAIDTKDSQTNSQLFNYFRDKAFPNLSARQLGVMPDLVLDMFINGYYLNVFKTQSTDVNRPYQDKDKRGGIFDAVFTRGDQTTLLTARHDLKNKGLNDISTIIKQELTEGRALALSHTYANVSISHVINLWGADFNAEGNLEAIYVTDSDANASIGMKKYFVGINAHGHVAISAKKIEGENIGAQVLGLFTLSSGKDIWQKLS

SEQ ID NO: 33 - protein, 312 aa, Streptococcus equi
DDYQRNATEAYAKEVPHQITSVWTKGVTPPEQFTQGEDVIHAPYLAHQGWYDITKAFDGKDNLLCGAATAGNMLHWWFDQNKTEIEAYLSKHPEKQKIIIRNQELFDLKAAIDTKDSQTNSQLFNYFRDKAFPNLSARQLGVMPDLVLDMFINGYYLNVFKTQSTDVNRPYQDKDKRGGIFDAVFTRGDQTTLLTARHDLKNKGLNDISTIIKQELTEGRALALSHTYANVSISHVINLWGADFNAEGNLEAIYVTDSDANASIGMKKYFVGINAHGHVAISAKKIEGENIGAQVLGLFTLSSGKDIWQKLS

SEQ ID NO: 34 - protein, 312 aa, Streptococcus equi
DDYQRNATEAYAKEVPHQITSVWTKGVTPPEQFTQGEDVIHAPYLANQGWYDITKAFDGKDNLLCGAATAGNMLHWWFDQNKTEIEAYLSKHPEKQKIIFRNQELFDLKEAIRTKDSQTNSQLFEYFRDKAFPYLSARQLGVMPDLVLDMFINGYYLNVFKTQSTDVKRPYQDKDKRGGIFDAVFTRGNQTTLLTARHDLKNKGLNDISTIIKEELTKGRALALSHTYANVSISHVINLWGADFNAEGNLEAIYVTDSDANASIGMKKYFVGINKHGHVAISAKKIEGENIGAQVLGLFTLSSGKDIWQKLN

SEQ ID NO: 35 - protein, 292 aa, Streptococcus equi
SVWTKGVTPPEQFTQGEDVIHAPYLAHQGWYDITKAFDGKDNLLCGAATAGNMLHWWFDQNKTEIEAYLSKHPEKQKIIFRNQELFDLKAAIDTKDSQTNSQLFNYFRDKAFPNLSARQLGVMPDLVLDMFINGYYLNVFKTQSTDVNRPYQDKDKRGGIFDAVFTRGNQTTLLTARHDLKNKGLNDISTIIKQELTEGRALALSHTYANVSISHVINLWGADFNAEGNLEAIYVTDSDANASIGMKKYFVGINAHGHVAISAKKIEGENIGAQVLGLFTLSSGKDIWQKLS

SEQ ID NO: 36 - protein, 312 aa, Streptococcus equi
DDYQRNATEAYAKEVPHQITSVWTKGVTPPEQFTQGEDVIHAPYLAHQGWYDITKAFDGADNLLCGAATAGNMLHWWFDQNKTEIEAYLSKHPEKQKIIFRNQELFDLKAAIDTKDSQTNSQLFNYFRDKAFPNLSARQLGVMPDLVLDMFINGYYLNVFKTQSTDVNRPYQDKDKRGGIFDAVFTRGNQTTLLTARHDLKNKGLNDISTIIKQELTEGRALALSHTYANVSISHVINLWGADFNAEGNLEAIYVTDSDANASIGMKKYFVGINAHGHVAISAKKIEGENIGAQVLGLFTLSSGKDIWQKLS

SEQ ID NO: 37 - protein, 292 aa, Streptococcus equi
SVWTKGVTPPEQFTQGEDVIHAPYLAHQGWYDITKAFDGADNLLCGAATAGNMLHWWFDQNKTEIEAYLSKHPEKQKIIFRNQELFDLKAAIDTKDSQTNSQLFNYFRDKAFPNLSARQLGVMPDLVLDMFINGYYLNVFKTQSTDVNRPYQDKDKRGGIFDAVFTRGNQTTLLTARHDLKNKGLNDISTIIKQELTEGRALALSHTYANVSISHVINLWGADFNAEGNLEAIYVTDSDANASIGMKKYFVGINAHGHVAISAKKIEGENIGAQVLGLFTLSSGKDIWQKLS

SEQ ID NO: 38 - protein, 312 aa, Streptococcus equi
DDYQRNATEAYAKEVPHQITSVWTKGVTPPEQFTQGEDVIHAPYLAHQGWYDITKAFDGKDNLLCGAATAGNMLHWWFDQNKTEIEAYLSKHPEKQKIIFRNQELFDLKAAIDTKDSQTNSQLFNYFRDKAFPNLSARQLGVMPDLVLDMFINGYYLNVFKTQSTDVNRPYQDKDKRGGIFDAVFTRGNQTTLLTARHDLKNKGLNDISTIIKQELTEGRALALSHTYANVSISHVINLWGADFNAEGNLEAIYVTDSDANASIGMKKYFVGINAHGHVAISAKKIEGENIGAQVLGLFTLSSGKDIWQKLS

SEQ ID NO: 39 - protein, 312 aa, Streptococcus equi
DDYQRNATEAYAKEVPHQITSVWTKGVTPLTPEQFTQGEDVFHAPYVANQGWYDITKAFDGKDNLLCGAATAGNMLHWWFDQNKDQIKRYLEEHPEKQKINFNGENMFDVKKAIDTKNHQLDSKLFNYFKEKAFPYLSAKHLGVFPDHVIDMFINGYRLSLTNHGPTPVKEGSKDPRGGIFDAVFTRGNQSKLLTSRHDFKNKNLNDISTIIKQELTKGKALGLSHTYANVRINHVINLWGADFNAEGNLEAIYVTDSDSNASIGMKKYFVGVNAHGHVAISAKKIEGENIGAQVLGLFTLSTGQDSWQKLS

SEQ ID NO: 40 - protein, 312 aa, Streptococcus equi
DDYQRNATEAYAKEVPHQITSVWTKGVTPLTPEQFTQGEDVFHAPYVANQGWYDITKAFDGKDNLLCGAATAGNMLHWWFDQNKDQIKRYLEEHPEKQKINFRGENMFDVKEAIRTKNHQLDSKLFEYFKEKAFPYLSAKHLGVFPDHVIDMFINGYRLSLTNHGPTPVKKGSKDPRGGIFDAVFTRGNQSKLLTSRHDFKNKNLNDISTIIKSELTNGKALGLSHTYANVRINHVINLWGADFNAEGNLEAIYVTDSDSNASIGMKKYFVGVNKHGHVAISAKKIEGENIGAQVLGLFTLSTGQDSWQKLN

SEQ ID NO: 41 - protein, 312 aa, Streptococcus equi
DDYQRNATEAYAKEVPHQITSVWTKGVTPLTPEQFTQGEDVFHAPYVANQGWYDITKTFNGKDDLLCGAATAGNMLHWWFDQNKDQIKRYLEEHPEKQKINFNGEQMFDVKEAIDTKNHQLDSKLFEYFKEKAFPYLSTKHLGVFPDHVIDMFINGYRLSLTNHGPTPVKEGSKDPRGGIFDAVFTRGNQSKLLTSRHDFKEKNLKEISDLIKQELTEGKALGLSHTYANVRINHVINLWGADFDAEGNLKAIYVTDSDSNASIGMKKYFVGVNAAGKVAISAKKIEGENIGAQVLGLFTLSTGQDSWNQTS

SEQ ID NO: 42 - protein, 312 aa, Streptococcus equi
DDYQRNATEAYAKEVPHQITSVWTKGVTPLTPEQFTQGEDVFHAPYVANQGWYDITKTFNGKDDLLCGAATAGNMLHWWFDQNKDQIKRYLEEHPEKQKINFRGEQMFDVKEAIRTKNHQLDSKLFEYFKEKAFPYLSTKHLGVFPDHVIDMFINGYRLSLTNHGPTPVKKGSKDPRGGIFDAVFTRGNQSKLLTSRHDFKEKNLKEISDLIKEELTKGKALGLSHTYANVRINHVINLWGADFDAEGNLKAIYVTDSDSNASIGMKKYFVGVNKAGKVAISAKKIEGENIGAQVLGLFTLSTGQDSWNQTN

SEQ ID NO: 43 - protein, 310 aa, Streptococcus equi
DDYQRNATEAYAKEVPHQITSVWTKGVTPPEQFTQGEDVIHAPYVANQGWYDITKAFDGKDNLLCGAATAGNMLHWWFDQNKDQIKRYLEEHPEKQKINFRGEQMFDVKKAIDTKNHQLDSKLFNYFKEKAFPGLSARRIGVFPDHVIDMFINGYRLSLTNHGPTPVKEGSKDPRGGIFDAVFTRGNQSKLLTSRHDFKNKNLNDISTIIKQELTKGKALGLSHTYANVSINHVINLWGADFNAEGNLEAIYVTDSDSNASIGMKKYFVGVNAHGHVAISAKKIEGENIGAQVLGLFTLSTGQDSWQKLS

SEQ ID NO: 44 - protein, 843 aa, Streptococcus pyogenes
MDKHLLVKRTLGCVCAATLMGAALATHHDSLNTVKAEEKTVQTGKTDQQVGAKLVQEIREGKRGPLYAGYFRTWHDRASTGIDGKQQHPENTMAEVPKEVDILFVFHDHTASDSPFWSELKDSYVHKLHQQGTALVQTIGVNELNGRTGLSKDYPDTPEGNKALAAAIVKAFVTDRGVDGLDIDIEHEFTNKRTPEEDARALNVFKEIAQLIGKNGSDKSKLLIMDTTLSVENNPIFKGIAEDLDYLLRQYYGSQGGEAEVDTINSDWNQYQNYIDASQFMIGFSFFEESASKGNLWFDVNEYDPNNPEKGKDIEGTRAKKYAEWQPSTGGLKAGIFSYAIDRDGVAHVPSTYKNRTSTNLQRHEVDNISHTDYTVSRKLKTLMTEDKRYDVIDQKDIPDPALREQIIQQVGQYKGDLERYNKTLVLTGDKIQNLKGLEKLSKLQKLELRQLSNVKEITPELLPESMKKDAELVMVGMTGLEKLNLSGLNRQTLDGIDVNSITHLTSFDISHNSLDLSEKSEDRKLLMTLMEQVSNHQKITVKNTAFENQKPKGYYPQTYDTKEGHYDVDNAEHDILTDFVFGTVTKRNTFIGDEEAFAIYKEGAVDGRQYVSKDYTYEAFRKDYKGYKVHLTASNLGETVTSKVTATTDETYLVDVSDGEKVVHHMKLNIGSGAIMMENLAKGAKVIGTSGDFEQAKKIFDGEKSDRFFTWGQTNWIAFDLGEINLAKEWRLFNAETNTEIKTDSSLNVAKGRLQILKDTTIDLEKMDIKNRKEYLSNDENWTDVAQMDDAKAIFNSKLSNVLSRYWRFCVDGGASSYYPQYTELQILGQRLSNDVANTLKD

SEQ ID NO: 45 - protein, 959 aa, Streptococcus pyogenes
EEKTVQVQKGLPSIDSLHYLSENSKKEFKEELSKAGQESQKVKEILAKAQQADKQAQELAKMKIPEKIPMKPLHGPLYGGYFRTWHDKTSDPTEKDKVNSMGELPKEVDLAFIFHDWTKDYSLFWKELATKHVPKLNKQGTRVIRTIPWRFLAGGDNSGIAEDTSKYPNTPEGNKALAKAIVDEYVYKYNLDGLDVDVEHDSIPKVDKKEDTAGVERSIQVFEEIGKLIGPKGVDKSRLFIMDSTYMADKNPLIERGAPYINLLLVQVYGSQGEKGGWEPVSNRPEKTMEERWQGYSKYIRPEQYMIGFSFYEENAQEGNLWYDINSRKDEDKANGINTDITGTRAERYARWQPKTGGVKGGIFSYAIDRDGVAHQPKKYAKQKEFKDATDNIFHSDYSVSKALKTVMLKDKSYDLIDEKDFPDKALREAVMAQVGTRKGDLERFNGTLRLDNPAIQSLEGLNKFKKLAQLDLIGLSRITKLDRSVLPANMKPGKDTLETVLETYKKDNKEEPATIPPVSLKVSGLTGLKELDLSGFDRETLAGLDAATLTSLEKVDISGNKLDLAPGTENRQIFDTMLSTISNHVGSNEQTVKFDKQKPTGHYPDTYGKTSLRLPVANEKVDLQSQLLFGTVTNQGTLINSEADYKAYQNHKIAGRSFVDSNYHYNNFKVSYENYTVKVTDSTLGTTTDKTLATDKEETYKVDFFSPADKTKAVHTAKVIVGDEKTMMVNLAEGATVIGGSADPVNARKVFDGQLGSETDNISLGWDSKQSIIFKLKEDGLIKHWRFFNDSARNPETTNKPIQEASLQIFNIKDYNLDNLLENPNKFDDEKYWITVDTYSAQGERATAFSNTLNNITSKYWRVVFDTKGDRYSSPVVPELQILGYPLPNADTIMKTVTTAKELSQQKDKFSQKMLDELKIKEMALETSLNSKIFDVTAINANAGVLKDCIEKRQLLKK

SEQ ID NO: 46 - protein, 995 aa, Streptococcus pyogenes
MDKHLLVKRTLGCVCAATLMGAALATHHDSLNTVKAEEKTVQVQKGLPSIDSLHYLSENSKKEFKEELSKAGQESQKVKEILAKAQQADKQAQELAKMKIPEKIPMKPLHGPLYGGYFRTWHDKTSDPTEKDKVNSMGELPKEVDLAFIFHDWTKDYSLFWKELATKHVPKLNKQGTRVIRTIPWRFLAGGDNSGIAEDTSKYPNTPEGNKALAKAIVDEYVYKYNLDGLDVDVEHDSIPKVDKKEDTAGVERSIQVFEEIGKLIGPKGVDKSRLFIMDSTYMADKNPLIERGAPYINLLLVQVYGSQGEKGGWEPVSNRPEKTMEERWQGYSKYIRPEQYMIGFSFYEENAQEGNLWYDINSRKDEDKANGINTDITGTRAERYARWQPKTGGVKGGIFSYAIDRDGVAHQPKKYAKQKEFKDATDNIFHSDYSVSKALKTVMLKDKSYDLIDEKDFPDKALREAVMAQVGTRKGDLERFNGTLRLDNPAIQSLEGLNKFKKLAQLDLIGLSRITKLDRSVLPANMKPGKDTLETVLETYKKDNKEEPATIPPVSLKVSGLTGLKELDLSGFDRETLAGLDAATLTSLEKVDISGNKLDLAPGTENRQIFDTMLSTISNHVGSNEQTVKFDKQKPTGHYPDTYGKTSLRLPVANEKVDLQSQLLFGTVTNQGTLINSEADYKAYQNHKIAGRSFVDSNYHYNNFKVSYENYTVKVTDSTLGTTTDKTLATDKEETYKVDFFSPADKTKAVHTAKVIVGDEKTMMVNLAEGATVIGGSADPVNARKVFDGQLGSETDNISLGWDSKQSIIFKLKEDGLIKHWRFFNDSARNPETTNKPIQEASLQIFNIKDYNLDNLLENPNKFDDEKYWITVDTYSAQGERATAFSNTLNNITSKYWRVVFDTKGDRYSSPVVPELQILGYPLPNADTIMKTVTTAKELSQQKDKFSQKMLDELKIKEMALETSLNSKIFDVTAINANAGVLKDCIEKRQLLKK

SEQ ID NO: 47 - protein, 995 aa, Streptococcus pyogenes; identical to SEQ ID NO: 46

SEQ ID NO: 48 - protein, 311 aa, Streptococcus pyogenes
MDSFSANQEIRYSEVTPYHVTSVWTKGVTPPANFTQGEDVFHAPYVANQGWYDITKTFNGKDDLLCGAATAGNMLHWWFDQNKDQIKRYLEEHPEKQKINFNGEQMFDVKEAIDTKNHQLDSKLFEYFKEKAFPYLSTKHLGVFPDHVIDMFINGYRLSLTNHGPTPVKEGSKDPRGGIFDAVFTRGDQSKLLTSRHDFKEKNLKEISDLIKKELTEGKALGLSHTYANVRINHVINLWGADFDSNGNLKAIYVTDSDSNASIGMKKYFVGVNSAGKVAISAKEIKEDNIGAQVLGLFTLSTGQDSWNQTN

SEQ ID NO: 49 - protein, 29 aa, synthetic construct
  REGION 1..29: note = Signal sequence
MRKRCYSTSAAVLAAVTLFVLSVDRGVIA

SEQ ID NO: 50 - protein, 29 aa, synthetic construct
  REGION 1..29: note = Signal sequence
MRKRCYSTSAAVLAAVTLFALSVDRGVIA

SEQ ID NO: 51 - protein, 29 aa, synthetic construct
  REGION 1..29: note = Signal sequence
MRKRCYSTSAVVLAAVTLFALSVDRGVIA

SEQ ID NO: 52 - DNA, 933 bp, Streptococcus pyogenes
  source 1..933: mol_type = other DNA
gatagtttttctgctaatcaagagattagatattcggaagtaacaccttatcacgttacttccgtttggaccaaaggagttactcctccagcaaacttcactcaaggtgaagatgtttttcacgctccttatgttgctaaccaaggatggtatgatattaccaaaacattcaatggaaaagacgatcttctttgcggggctgccacagcagggaatatgcttcactggtggttcgatcaaaacaaagaccaaattaaacgttatttggaagagcatccagaaaagcaaaaaataaacttcaatggcgaacagatgtttgacgtaaaagaagctatcgacactaaaaaccaccagctagatagtaaattatttgaatattttaaagaaaaagctttcccttatctatctactaaacacctaggagttttccctgatcatgtaattgatatgttcattaacggctaccgccttagtctaactaaccacggtccaacgccagtaaaagaaggtagtaaagatccccgaggtggtatttttgacgccgtatttacaagaggtgatcaaagtaagctattgacaagtcgtcatgattttaaagaaaaaaatctcaaagaaatcagtgatctcattaagaaagagttaaccgaaggcaaggctctaggcctatcacacacctacgctaacgtacgcatcaaccatgttataaacctgtggggagctgactttgattctaacgggaaccttaaagctatttatgtaacagactctgatagtaatgcatctattggtatgaagaaatactttgttggtgttaattccgctggaaaagtagctatttctgctaaagaaataaaagaagataatattggtgctcaagtactagggttatttacactttcaacagggcaagatagttggaatcagaccaattaa